European Patent Specification EP 3 585 445 B1, published February 7, 2024. Title: Humanized Model of Kidney and Liver Disorders. Applicant: Regeneron Pharmaceuticals, Inc. The sequence listing filed with the application follows.

SEQUENCE LISTING (27 sequences)

SEQ ID NO: 1 - DNA, 22 bp, Artificial Sequence
  synthetic oligonucleotide
ggcctgattacatggacctgtc

SEQ ID NO: 2 - DNA, 19 bp, Artificial Sequence
  synthetic oligonucleotide
cccaggcttggctggaatg

SEQ ID NO: 3 - DNA, 22 bp, Artificial Sequence
  synthetic oligonucleotide
tgtccactctggaagcccaggc

SEQ ID NO: 4 - DNA, 20 bp, Artificial Sequence
  synthetic oligonucleotide
gccaggagaggaagctggag

SEQ ID NO: 5 - DNA, 21 bp, Artificial Sequence
  synthetic oligonucleotide
tggctcagcagtaaagaacac

SEQ ID NO: 6 - DNA, 24 bp, Artificial Sequence
  synthetic oligonucleotide
acagattgctgtgagctgcccaaa

SEQ ID NO: 7 - DNA, 19 bp, Artificial Sequence
  synthetic oligonucleotide
ggtggagaggctattcggc

SEQ ID NO: 8 - DNA, 17 bp, Artificial Sequence
  synthetic oligonucleotide
gaacacggcggcatcag

SEQ ID NO: 9 - DNA, 23 bp, Artificial Sequence
  synthetic oligonucleotide
tgggcacaacagacaatcggctg

SEQ ID NO: 10 - DNA, 19 bp, Artificial Sequence
  synthetic oligonucleotide
gccagcctagcctacttca

SEQ ID NO: 11 - DNA, 18 bp, Artificial Sequence
  synthetic oligonucleotide
gccacccatcccagttct

SEQ ID NO: 12 - DNA, 23 bp, Artificial Sequence
  synthetic oligonucleotide
cagcccaggccctttagattgca

SEQ ID NO: 13 - DNA, 24 bp, Artificial Sequence
  synthetic oligonucleotide
tacggtgttaggttcactattggt

SEQ ID NO: 14 - DNA, 21 bp, Artificial Sequence
  synthetic oligonucleotide
gtcgccagcagtctcatacag

SEQ ID NO: 15 - DNA, 17 bp, Artificial Sequence
  synthetic oligonucleotide
tgcggccgatcttagcc

SEQ ID NO: 16 - DNA, 18 bp, Artificial Sequence
  synthetic oligonucleotide
ttgaccgattccttgcgg

SEQ ID NO: 17 - DNA, 25 bp, Artificial Sequence
  synthetic oligonucleotide
gggcctcctaagtttgttgagtatc

SEQ ID NO: 18 - DNA, 22 bp, Artificial Sequence
  synthetic oligonucleotide
cagggctggttccctagaaatc

SEQ ID NO: 19 - DNA, 23 bp, Artificial Sequence
  synthetic oligonucleotide
tacaatagcaggcacagcaccca

SEQ ID NO: 20 - DNA, 20 bp, Artificial Sequence
  synthetic oligonucleotide
ggctgagagtgggagtcatg

SEQ ID NO: 21 - DNA, 21 bp, Artificial Sequence
  synthetic oligonucleotide
gcacttgccaatgccattatc

SEQ ID NO: 22 - DNA, 23 bp, Artificial Sequence
  synthetic oligonucleotide
ctgctgtcctgcccatgtggttg

SEQ ID NO: 23 - DNA, 22 bp, Artificial Sequence
  synthetic oligonucleotide
cgaatgccaagacgaagagaac

SEQ ID NO: 24 - DNA, 20 bp, Artificial Sequence
  synthetic oligonucleotide
gggcacccaaagacaaccat

SEQ ID NO: 25 - DNA, 24 bp, Artificial Sequence
  synthetic oligonucleotide
cagaaacaatgccaggacctcggc

SEQ ID NO: 26 - DNA, 21 bp, Artificial Sequence
  synthetic oligonucleotide
agtgggcatcccttgccaggc

SEQ ID NO: 27 - DNA, 21 bp, Artificial Sequence
  synthetic oligonucleotide
acgagcgggttcggcccattc